European Patent Application EP 4 570 263 A1, published June 18, 2025. Title: TCRs recognizing G12V mutated RAS and uses thereof. Applicant: Genovie AB. The sequence listing filed with the application follows.

SEQUENCE LISTING (122 sequences)

SEQ ID NO: 1 - protein, 10 aa, Homo sapiens
VVVGAVGVGK

SEQ ID NO: 2 - protein, 9 aa, Homo sapiens
VVGAVGVGK

SEQ ID NO: 3 - protein, 10 aa, Homo sapiens
VVVGAGGVGK

SEQ ID NO: 4 - protein, 9 aa, Homo sapiens
VVGAGGVGK

SEQ ID NO: 5 - protein, 24 aa, Homo sapiens
TEYKLVVVGAVGVGKSALTIQLIQ

SEQ ID NO: 6 - protein, 188 aa, Homo sapiens
MTEYKLVVVGAVGVGKSALTIQLIQNHFVDEYDPTIEMSYRKQVVIDGETCLLDILDTAGQEEYSAMRDQYMRTGEGFLCVFAINNTKSFEDIHHYREQIKRVKDSEDVPMVLVGNKCDLPSRTVDTKQAQDLARSYGIPFIETSAKTRQGVDDAFYTLVREIRKHKEKMSKDGKKKKKKSKTKCVIM

SEQ ID NO: 7 - protein, 11 aa, Homo sapiens
GTGTQLKVELN

SEQ ID NO: 8 - protein, 10 aa, Homo sapiens
GDGTRLSILE

SEQ ID NO: 9 - protein, 11 aa, Homo sapiens
GAGTRLFVKAN

SEQ ID NO: 10 - protein, 10 aa, Homo sapiens
GSGTRLTVVE

SEQ ID NO: 11 - protein, 11 aa, Homo sapiens
GEGTQLTVNPD

SEQ ID NO: 12 - protein, 10 aa, Homo sapiens
GPGTRLTVTE

SEQ ID NO: 13 - protein, 11 aa, Homo sapiens
GKGTHLIIQPY

SEQ ID NO: 14 - protein, 11 aa, Homo sapiens
GTGTRLTVIPY

SEQ ID NO: 15 - protein, 11 aa, Homo sapiens
GAGTRLAVHPY

SEQ ID NO: 16 - protein, 10 aa, Homo sapiens
GEGSRLTVLE

SEQ ID NO: 17 - protein, 10 aa, Homo sapiens
GQGTRLTVVE

SEQ ID NO: 18 - protein, 46 aa, Homo sapiens
MLTASLLRAVIASICVVSSMAQKVTQAQTEISVVEKEDVTLDCVYE

SEQ ID NO: 19 - protein, 45 aa, Homo sapiens
MGPGLLCWVLLCLLGAGPVDAGVTQSPTHLIKTRGQQVTLRCSPI

SEQ ID NO: 20 - protein, 48 aa, Homo sapiens
MMKSLRVLLVILWLQLSWVWSQQKEVEQNSGPLSVPEGAIASLNCTYS

SEQ ID NO: 21 - protein, 45 aa, Homo sapiens
MSNQVLCCVVLCFLGANTVDGGITQSPKYLFRKEGQNVTLSCEQN

SEQ ID NO: 22 - protein, 46 aa, Homo sapiens
MTRVSLLWAVVVSTCLESGMAQTVTQSQPEMSVQEAETVTLSCTYD

SEQ ID NO: 23 - protein, 41 aa, Homo sapiens
MLSLLLLLLGLGSVFSAVISQKPSRDICQRGTSLTIQCQVD

SEQ ID NO: 24 - protein, 46 aa, Homo sapiens
METLLGVSLVILWLQLARVNSQQGEEDPQALSIQEGENATMNCSYK

SEQ ID NO: 25 - protein, 45 aa, Homo sapiens
MSPIFTCITILCLLAAGSPGEEVAQTPKHLVRGEGQKAKLYCAPI

SEQ ID NO: 26 - protein, 46 aa, Homo sapiens
MKTFAGFSFLFLWLQLDCMSRGEDVEQSLFLSVREGDSSVINCTYT

SEQ ID NO: 27 - protein, 45 aa, Homo sapiens
MTIRLLCYMGFYFLGAGLMEADIYQTPRYLVIGTGKKITLECSQT

SEQ ID NO: 28 - protein, 42 aa, Homo sapiens
MWGVFLLYVSMKMGGTTGQNIDQPTEMTATEGAIVQINCTYQ

SEQ ID NO: 29 - protein, 45 aa, Homo sapiens
MGPQLLGYVVLCLLGAGPLEAQVTQNPRYLITVTGKKLTVTCSQN

SEQ ID NO: 30 - protein, 45 aa, Homo sapiens
MGTRLLCWAALCLLGAELTEAGVAQSPRYKIIEKRQSVAFWCNPI

SEQ ID NO: 31 - protein, 45 aa, Homo sapiens
MGFRLLCCVAFCLLGAGPVDSGVTQTPKHLITATGQRVTLRCSPR

SEQ ID NO: 32 - protein, 17 aa, Homo sapiens
LFWYKQPPSGELVFLIR

SEQ ID NO: 33 - protein, 17 aa, Homo sapiens
VSWYQQVLGQGPQFIFQ

SEQ ID NO: 34 - protein, 17 aa, Homo sapiens
FFWYRQYSGKSPELIMF

SEQ ID NO: 35 - protein, 17 aa, Homo sapiens
MYWYRQDPGQGLRLIYY

SEQ ID NO: 36 - protein, 17 aa, Homo sapiens
LFWYKQPPSRQMILVIR

SEQ ID NO: 37 - protein, 17 aa, Homo sapiens
MFWYRQQPGQSLTLIAT

SEQ ID NO: 38 - protein, 17 aa, Homo sapiens
LQWYRQNSGRGLVHLIL

SEQ ID NO: 39 - protein, 17 aa, Homo sapiens
VFWYQQVLKNEFKFLIS

SEQ ID NO: 40 - protein, 17 aa, Homo sapiens
LYWYKQEPGAGLQLLTY

SEQ ID NO: 41 - protein, 17 aa, Homo sapiens
MYWYQQDPGMELHLIHY

SEQ ID NO: 42 - protein, 17 aa, Homo sapiens
LFWYQQHAGEAPTFLSY

SEQ ID NO: 43 - protein, 17 aa, Homo sapiens
MSWYRQDPGLGLRQIYY

SEQ ID NO: 44 - protein, 17 aa, Homo sapiens
LYWYQQILGQGPKLLIQ

SEQ ID NO: 45 - protein, 17 aa, Homo sapiens
VYWYQQSLDQGLQFLIQ

SEQ ID NO: 46 - protein, 33 aa, Homo sapiens
EISGRYSWNFQKSTSSFNFTITASQVVDSAVYF

SEQ ID NO: 47 - protein, 36 aa, Homo sapiens
RGRGNFPDRFSARQFPNYSSELNVNALLLGDSALYL

SEQ ID NO: 48 - protein, 33 aa, Homo sapiens
KEDGRFTAQLNKASQYVSLLIRDSQPSDSATYL

SEQ ID NO: 49 - protein, 36 aa, Homo sapiens
FQKGDIAEGYSVSREKKESFPLTVTSAQKNPTAFYL

SEQ ID NO: 50 - protein, 33 aa, Homo sapiens
ATENRFSVNFQKAAKSFSLKISDSQLGDTAMYF

SEQ ID NO: 51 - protein, 37 aa, Homo sapiens
TYESGFVIDKFPISRPNLTFSTLTVSNMSPEDSSIYL

SEQ ID NO: 52 - protein, 33 aa, Homo sapiens
KHSGRLRVTLDTSKKSSSLLITASRAADTASYF

SEQ ID NO: 53 - protein, 37 aa, Homo sapiens
FDETGMPKERFSAKCLPNSPCSLEIQATKLEDSAVYF

SEQ ID NO: 54 - protein, 33 aa, Homo sapiens
KQDQRLTVLLNKKDKHLSLRIADTQTGDSAIYF

SEQ ID NO: 55 - protein, 36 aa, Homo sapiens
TEKGDLSSESTVSRIRTEHFPLTLESARPSHTSQYL

SEQ ID NO: 56 - protein, 33 aa, Homo sapiens
EEKGRFSSFLSRSKGYSYLLLKELQMKDSASYL

SEQ ID NO: 57 - protein, 36 aa, Homo sapiens
TDKGDVPEGYKVSRKEKRNFPLILESPSPNQTSLYF

SEQ ID NO: 58 - protein, 37 aa, Homo sapiens
VDDSQLPKDRFSAERLKGVDSTLKIQPAKLEDSAVYL

SEQ ID NO: 59 - protein, 36 aa, Homo sapiens
RAKGNILERFSAQQFPDLHSELNLSSLELGDSALYF

SEQ ID NO: 60 - protein, 7 aa, Homo sapiens
TRDTTYY

SEQ ID NO: 61 - protein, 5 aa, Homo sapiens
SGHKS

SEQ ID NO: 62 - protein, 6 aa, Homo sapiens
DRGSQS

SEQ ID NO: 63 - protein, 5 aa, Homo sapiens
LNHDA

SEQ ID NO: 64 - protein, 7 aa, Homo sapiens
TSENNYY

SEQ ID NO: 65 - protein, 5 aa, Homo sapiens
SQVTM

SEQ ID NO: 66 - protein, 5 aa, Homo sapiens
TSINN

SEQ ID NO: 67 - protein, 5 aa, Homo sapiens
KGHSY

SEQ ID NO: 68 - protein, 6 aa, Homo sapiens
DSSSTY

SEQ ID NO: 69 - protein, 5 aa, Homo sapiens
MGHDK

SEQ ID NO: 70 - protein, 6 aa, Homo sapiens
TSGFNG

SEQ ID NO: 71 - protein, 5 aa, Homo sapiens
MNHEY

SEQ ID NO: 72 - protein, 5 aa, Homo sapiens
SGHAT

SEQ ID NO: 73 - protein, 5 aa, Homo sapiens
SGDLS

SEQ ID NO: 74 - protein, 8 aa, Homo sapiens
RNSFDEQN

SEQ ID NO: 75 - protein, 6 aa, Homo sapiens
YYEKEE

SEQ ID NO: 76 - protein, 6 aa, Homo sapiens
IYSNGD

SEQ ID NO: 77 - protein, 6 aa, Homo sapiens
SQIVND

SEQ ID NO: 78 - protein, 8 aa, Homo sapiens
QEAYKQQN

SEQ ID NO: 79 - protein, 7 aa, Homo sapiens
ANQGSEA

SEQ ID NO: 80 - protein, 7 aa, Homo sapiens
IRSNERE

SEQ ID NO: 81 - protein, 6 aa, Homo sapiens
FQNENV

SEQ ID NO: 82 - protein, 7 aa, Homo sapiens
IFSNMDM

SEQ ID NO: 83 - protein, 6 aa, Homo sapiens
SYGVNS

SEQ ID NO: 84 - protein, 6 aa, Homo sapiens
NVLDGL

SEQ ID NO: 85 - protein, 6 aa, Homo sapiens
SMNVEV

SEQ ID NO: 86 - protein, 6 aa, Homo sapiens
FQNNGV

SEQ ID NO: 87 - protein, 6 aa, Homo sapiens
YYNGEE

SEQ ID NO: 88 - protein, 14 aa, Homo sapiens
CALILTGGGNKLTF

SEQ ID NO: 89 - protein, 15 aa, Homo sapiens
CASSPSGDYDQPQHF

SEQ ID NO: 90 - protein, 12 aa, Homo sapiens
CAVNTGGFKTIF

SEQ ID NO: 91 - protein, 12 aa, Homo sapiens
CASLGGDYGYTF

SEQ ID NO: 92 - protein, 15 aa, Homo sapiens
CAFMNGETSGSRLTF

SEQ ID NO: 93 - protein, 13 aa, Homo sapiens
CSVVGRGTYEQYF

SEQ ID NO: 94 - protein, 15 aa, Homo sapiens
CATDASGGGADGLTF

SEQ ID NO: 95 - protein, 12 aa, Homo sapiens
CASSQWNQPQHF

SEQ ID NO: 96 - protein, 11 aa, Homo sapiens
CAGSGANNLFF

SEQ ID NO: 97 - protein, 15 aa, Homo sapiens
CASSELGQVDYGYTF

SEQ ID NO: 98 - protein, 13 aa, Homo sapiens
CAALSGGYNKLIF

SEQ ID NO: 99 - protein, 14 aa, Homo sapiens
CASSLVKGAGELFF

SEQ ID NO: 100 - protein, 14 aa, Homo sapiens
CATDGNTGGFKTIF

SEQ ID NO: 101 - protein, 13 aa, Homo sapiens
CASSLETSYEQYF

SEQ ID NO: 102 - protein, 14 aa, Homo sapiens
CAVTSRGGADGLTF

SEQ ID NO: 103 - protein, 14 aa, Homo sapiens
CASSAYREDTEAFF

SEQ ID NO: 104 - protein, 140 aa, Homo sapiens
IQNPDPAVYQLRDSKSSDKSVCLFTDFDSQTNVSQSKDSDVYITDKTVLDMRSMDFKSNSAVAWSNKSDFACANAFNNSIIPEDTFFPSPESSCDVKLVEKSFETDTNLNFQNLSVIGFRILLLKVAGFNLLMTLRLWSS

SEQ ID NO: 105 - protein, 178 aa, Homo sapiens
DLNKVFPPEVAVFEPSEAEISHTQKATLVCLATGFYPDHVELSWWVNGKEVHSGVSTDPQPLKEQPALNDSRYCLSSRLRVSATFWQNPRNHFRCQVQFYGLSENDEWTQDRAKPVTQIVSAEAWGRADCGFTSESYQQGVLSATILYEILLGKATLYAVLVSALVLMAMVKRKDSRG

SEQ ID NO: 106 - protein, 178 aa, Homo sapiens
DLKNVFPPEVAVFEPSEAEISHTQKATLVCLATGFYPDHVELSWWVNGKEVHSGVSTDPQPLKEQPALNDSRYCLSSRLRVSATFWQNPRNHFRCQVQFYGLSENDEWTQDRAKPVTQIVSAEAWGRADCGFTSESYQQGVLSATILYEILLGKATLYAVLVSALVLMAMVKRKDSRG

SEQ ID NO: 107 - protein, 276 aa, Homo sapiens
MLTASLLRAVIASICVVSSMAQKVTQAQTEISVVEKEDVTLDCVYETRDTTYYLFWYKQPPSGELVFLIRRNSFDEQNEISGRYSWNFQKSTSSFNFTITASQVVDSAVYFCALILTGGGNKLTFGTGTQLKVELNIQNPDPAVYQLRDSKSSDKSVCLFTDFDSQTNVSQSKDSDVYITDKTVLDMRSMDFKSNSAVAWSNKSDFACANAFNNSIIPEDTFFPSPESSCDVKLVEKSFETDTNLNFQNLSVIGFRILLLKVAGFNLLMTLRLWSS

SEQ ID NO: 108 - protein, 312 aa, Homo sapiens
MGPGLLCWVLLCLLGAGPVDAGVTQSPTHLIKTRGQQVTLRCSPISGHKSVSWYQQVLGQGPQFIFQYYEKEERGRGNFPDRFSARQFPNYSSELNVNALLLGDSALYLCASSPSGDYDQPQHFGDGTRLSILEDLNKVFPPEVAVFEPSEAEISHTQKATLVCLATGFYPDHVELSWWVNGKEVHSGVSTDPQPLKEQPALNDSRYCLSSRLRVSATFWQNPRNHFRCQVQFYGLSENDEWTQDRAKPVTQIVSAEAWGRADCGFTSESYQQGVLSATILYEILLGKATLYAVLVSALVLMAMVKRKDSRG

SEQ ID NO: 109 - protein, 273 aa, Homo sapiens
MMKSLRVLLVILWLQLSWVWSQQKEVEQNSGPLSVPEGAIASLNCTYSDRGSQSFFWYRQYSGKSPELIMFIYSNGDKEDGRFTAQLNKASQYVSLLIRDSQPSDSATYLCAVNTGGFKTIFGAGTRLFVKANIQNPDPAVYQLRDSKSSDKSVCLFTDFDSQTNVSQSKDSDVYITDKTVLDMRSMDFKSNSAVAWSNKSDFACANAFNNSIIPEDTFFPSPESSCDVKLVEKSFETDTNLNFQNLSVIGFRILLLKVAGFNLLMTLRLWSS

SEQ ID NO: 110 - protein, 309 aa, Homo sapiens
MSNQVLCCVVLCFLGANTVDGGITQSPKYLFRKEGQNVTLSCEQNLNHDAMYWYRQDPGQGLRLIYYSQIVNDFQKGDIAEGYSVSREKKESFPLTVTSAQKNPTAFYLCASLGGDYGYTFGSGTRLTVVEDLNKVFPPEVAVFEPSEAEISHTQKATLVCLATGFYPDHVELSWWVNGKEVHSGVSTDPQPLKEQPALNDSRYCLSSRLRVSATFWQNPRNHFRCQVQFYGLSENDEWTQDRAKPVTQIVSAEAWGRADCGFTSESYQQGVLSATILYEILLGKATLYAVLVSALVLMAMVKRKDSRG

SEQ ID NO: 111 - protein, 277 aa, Homo sapiens
MTRVSLLWAVVVSTCLESGMAQTVTQSQPEMSVQEAETVTLSCTYDTSENNYYLFWYKQPPSRQMILVIRQEAYKQQNATENRFSVNFQKAAKSFSLKISDSQLGDTAMYFCAFMNGETSGSRLTFGEGTQLTVNPDIQNPDPAVYQLRDSKSSDKSVCLFTDFDSQTNVSQSKDSDVYITDKTVLDMRSMDFKSNSAVAWSNKSDFACANAFNNSIIPEDTFFPSPESSCDVKLVEKSFETDTNLNFQNLSVIGFRILLLKVAGFNLLMTLRLWSS

SEQ ID NO: 112 - protein, 308 aa, Homo sapiens
MLSLLLLLLGLGSVFSAVISQKPSRDICQRGTSLTIQCQVDSQVTMMFWYRQQPGQSLTLIATANQGSEATYESGFVIDKFPISRPNLTFSTLTVSNMSPEDSSIYLCSVVGRGTYEQYFGPGTRLTVTEDLKNVFPPEVAVFEPSEAEISHTQKATLVCLATGFYPDHVELSWWVNGKEVHSGVSTDPQPLKEQPALNDSRYCLSSRLRVSATFWQNPRNHFRCQVQFYGLSENDEWTQDRAKPVTQIVSAEAWGRADCGFTSESYQQGVLSATILYEILLGKATLYAVLVSALVLMAMVKRKDSRG

SEQ ID NO: 113 - protein, 274 aa, Homo sapiens
METLLGVSLVILWLQLARVNSQQGEEDPQALSIQEGENATMNCSYKTSINNLQWYRQNSGRGLVHLILIRSNEREKHSGRLRVTLDTSKKSSSLLITASRAADTASYFCATDASGGGADGLTFGKGTHLIIQPYIQNPDPAVYQLRDSKSSDKSVCLFTDFDSQTNVSQSKDSDVYITDKTVLDMRSMDFKSNSAVAWSNKSDFACANAFNNSIIPEDTFFPSPESSCDVKLVEKSFETDTNLNFQNLSVIGFRILLLKVAGFNLLMTLRLWSS

SEQ ID NO: 114 - protein, 310 aa, Homo sapiens
MSPIFTCITILCLLAAGSPGEEVAQTPKHLVRGEGQKAKLYCAPIKGHSYVFWYQQVLKNEFKFLISFQNENVFDETGMPKERFSAKCLPNSPCSLEIQATKLEDSAVYFCASSQWNQPQHFGDGTRLSILEDLNKVFPPEVAVFEPSEAEISHTQKATLVCLATGFYPDHVELSWWVNGKEVHSGVSTDPQPLKEQPALNDSRYCLSSRLRVSATFWQNPRNHFRCQVQFYGLSENDEWTQDRAKPVTQIVSAEAWGRADCGFTSESYQQGVLSATILYEILLGKATLYAVLVSALVLMAMVKRKDSRG

SEQ ID NO: 115 - protein, 271 aa, Homo sapiens
MKTFAGFSFLFLWLQLDCMSRGEDVEQSLFLSVREGDSSVINCTYTDSSSTYLYWYKQEPGAGLQLLTYIFSNMDMKQDQRLTVLLNKKDKHLSLRIADTQTGDSAIYFCAGSGANNLFFGTGTRLTVIPYIQNPDPAVYQLRDSKSSDKSVCLFTDFDSQTNVSQSKDSDVYITDKTVLDMRSMDFKSNSAVAWSNKSDFACANAFNNSIIPEDTFFPSPESSCDVKLVEKSFETDTNLNFQNLSVIGFRILLLKVAGFNLLMTLRLWSS

SEQ ID NO: 116 - protein, 312 aa, Homo sapiens
MTIRLLCYMGFYFLGAGLMEADIYQTPRYLVIGTGKKITLECSQTMGHDKMYWYQQDPGMELHLIHYSYGVNSTEKGDLSSESTVSRIRTEHFPLTLESARPSHTSQYLCASSELGQVDYGYTFGSGTRLTVVEDLNKVFPPEVAVFEPSEAEISHTQKATLVCLATGFYPDHVELSWWVNGKEVHSGVSTDPQPLKEQPALNDSRYCLSSRLRVSATFWQNPRNHFRCQVQFYGLSENDEWTQDRAKPVTQIVSAEAWGRADCGFTSESYQQGVLSATILYEILLGKATLYAVLVSALVLMAMVKRKDSRG

SEQ ID NO: 117 - protein, 268 aa, Homo sapiens
MWGVFLLYVSMKMGGTTGQNIDQPTEMTATEGAIVQINCTYQTSGFNGLFWYQQHAGEAPTFLSYNVLDGLEEKGRFSSFLSRSKGYSYLLLKELQMKDSASYLCAALSGGYNKLIFGAGTRLAVHPYIQNPDPAVYQLRDSKSSDKSVCLFTDFDSQTNVSQSKDSDVYITDKTVLDMRSMDFKSNSAVAWSNKSDFACANAFNNSIIPEDTFFPSPESSCDVKLVEKSFETDTNLNFQNLSVIGFRILLLKVAGFNLLMTLRLWSS

SEQ ID NO: 118 - protein, 311 aa, Homo sapiens
MGPQLLGYVVLCLLGAGPLEAQVTQNPRYLITVTGKKLTVTCSQNMNHEYMSWYRQDPGLGLRQIYYSMNVEVTDKGDVPEGYKVSRKEKRNFPLILESPSPNQTSLYFCASSLVKGAGELFFGEGSRLTVLEDLKNVFPPEVAVFEPSEAEISHTQKATLVCLATGFYPDHVELSWWVNGKEVHSGVSTDPQPLKEQPALNDSRYCLSSRLRVSATFWQNPRNHFRCQVQFYGLSENDEWTQDRAKPVTQIVSAEAWGRADCGFTSESYQQGVLSATILYEILLGKATLYAVLVSALVLMAMVKRKDSRG

SEQ ID NO: 119 - protein, 273 aa, Homo sapiens
METLLGVSLVILWLQLARVNSQQGEEDPQALSIQEGENATMNCSYKTSINNLQWYRQNSGRGLVHLILIRSNEREKHSGRLRVTLDTSKKSSSLLITASRAADTASYFCATDGNTGGFKTIFGAGTRLFVKANIQNPDPAVYQLRDSKSSDKSVCLFTDFDSQTNVSQSKDSDVYITDKTVLDMRSMDFKSNSAVAWSNKSDFACANAFNNSIIPEDTFFPSPESSCDVKLVEKSFETDTNLNFQNLSVIGFRILLLKVAGFNLLMTLRLWSS

SEQ ID NO: 120 - protein, 311 aa, Homo sapiens
MGTRLLCWAALCLLGAELTEAGVAQSPRYKIIEKRQSVAFWCNPISGHATLYWYQQILGQGPKLLIQFQNNGVVDDSQLPKDRFSAERLKGVDSTLKIQPAKLEDSAVYLCASSLETSYEQYFGPGTRLTVTEDLKNVFPPEVAVFEPSEAEISHTQKATLVCLATGFYPDHVELSWWVNGKEVHSGVSTDPQPLKEQPALNDSRYCLSSRLRVSATFWQNPRNHFRCQVQFYGLSENDEWTQDRAKPVTQIVSAEAWGRADCGFTSESYQQGVLSATILYEILLGKATLYAVLVSALVLMAMVKRKDSRG

SEQ ID NO: 121 - protein, 275 aa, Homo sapiens
MMKSLRVLLVILWLQLSWVWSQQKEVEQNSGPLSVPEGAIASLNCTYSDRGSQSFFWYRQYSGKSPELIMFIYSNGDKEDGRFTAQLNKASQYVSLLIRDSQPSDSATYLCAVTSRGGADGLTFGKGTHLIIQPYIQNPDPAVYQLRDSKSSDKSVCLFTDFDSQTNVSQSKDSDVYITDKTVLDMRSMDFKSNSAVAWSNKSDFACANAFNNSIIPEDTFFPSPESSCDVKLVEKSFETDTNLNFQNLSVIGFRILLLKVAGFNLLMTLRLWSS

SEQ ID NO: 122 - protein, 311 aa, Homo sapiens
MGFRLLCCVAFCLLGAGPVDSGVTQTPKHLITATGQRVTLRCSPRSGDLSVYWYQQSLDQGLQFLIQYYNGEERAKGNILERFSAQQFPDLHSELNLSSLELGDSALYFCASSAYREDTEAFFGQGTRLTVVEDLKNVFPPEVAVFEPSEAEISHTQKATLVCLATGFYPDHVELSWWVNGKEVHSGVSTDPQPLKEQPALNDSRYCLSSRLRVSATFWQNPRNHFRCQVQFYGLSENDEWTQDRAKPVTQIVSAEAWGRADCGFTSESYQQGVLSATILYEILLGKATLYAVLVSALVLMAMVKRKDSRG